European Patent Application EP 4 245 776 A1, published September 20, 2023. Title: FUSION PROTEIN OF HUMAN SERUM ALBUMIN AND INTERLEUKIN-2, AND USE THEREOF. Applicant: SINOBIOTECH (TIANJIN) LTD. FORTUNEROCK (CHINA) CO., LTD. BEIJING BIO-FORNTUNE, LTD. TIANJIN SINOBIOTECH, LTD. The sequence listing filed with the application follows.

SEQUENCE LISTING (14 sequences)

SEQ ID NO: 1 - protein, 718 aa, rHSA/IL-2 fusion, 9222
DAHKSEVAHRFKDLGEENFKALVLIAFAQYLQQCPFEDHVKLVNEVTEFAKTCVADESAENCDKSLHTLFGDKLCTVATLRETYGEMADCCAKQEPERNECFLQHKDDNPNLPRLVRPEVDVMCTAFHDNEETFLKKYLYEIARRHPYFYAPELLFFAKRYKAAFTECCQAADKAACLLPKLDELRDEGKASSAKQRLKCASLQKFGERAFKAWAVARLSQRFPKAEFAEVSKLVTDLTKVHTECCHGDLLECADDRADLAKYICENQDSISSKLKECCEKPLLEKSHCIAEVENDEMPADLPSLAADFVESKDVCKNYAEAKDVFLGMFLYEYARRHPDYSVVLLLRLAKTYETTLEKCCAAADPHECYAKVFDEFKPLVEEPQNLIKQNCELFEQLGEYKFQNALLVRYTKKVPQVSTPTLVEVSRNLGKVGSKCCKHPEAKRMPCAEDYLSVVLNQLCVLHEKTPVSDRVTKCCTESLVNRRPCFSALEVDETYVPKEFNAETFTFHADICTLSEKERQIKKQTALVELVKHKPKATKEQLKAVMDDFAAFVEKCCKADDKETCFAEEGKKLVAASQAALGLAPTSSSTKKTQLQLEHLLLDLQMILNGINNYKNPKLTRMLTFKFYMPKKATELKHLQCLEEELKPLEEVLNLAQSKNFHLRPRDLISNINVIVLELKGSETTFMCEYADETATIVEFLNRWITFCQSIISTLT

SEQ ID NO: 2 - DNA, 2232 bp, rHSA/IL-2 fusion, 9222
atgaagtgggtaacctttatttcccttctttttctctttagctcggcttattccaggggtgtgtttcgtcgagatgcacacaagagtgaggttgctcatcggtttaaagatttgggagaagaaaatttcaaagccttggtgttgattgcctttgctcagtatcttcagcagtgtccatttgaagatcatgtaaaattagtgaatgaagtaactgaatttgcaaaaacatgtgttgctgatgagtcagctgaaaattgtgacaaatcacttcataccctttttggagacaaattatgcacagttgcaactcttcgtgaaacctatggtgaaatggctgactgctgtgcaaaacaagaacctgagagaaatgaatgcttcttgcaacacaaagatgacaacccaaacctcccccgattggtgagaccagaggttgatgtgatgtgcactgcttttcatgacaatgaagagacatttttgaaaaaatacttatatgaaattgccagaagacatccttacttttatgccccggaactccttttctttgctaaaaggtataaagctgcttttacagaatgttgccaagctgctgataaagctgcctgcctgttgccaaagctcgatgaacttcgggatgaagggaaggcttcgtctgccaaacagagactcaagtgtgccagtctccaaaaatttggagaaagagctttcaaagcatgggcagtagctcgcctgagccagagatttcccaaagctgagtttgcagaagtttccaagttagtgacagatcttaccaaagtccacacggaatgctgccatggagatctgcttgaatgtgctgatgacagggcggaccttgccaagtatatctgtgaaaatcaagattcgatctccagtaaactgaaggaatgctgtgaaaaacctctgttggaaaaatcccactgcattgccgaagtggaaaatgatgagatgcctgctgacttgccttcattagctgctgattttgttgaaagtaaggatgtttgcaaaaactatgctgaggcaaaggatgtcttcctgggcatgtttttgtatgaatatgcaagaaggcatcctgattactctgtcgtgctgctgctgagacttgccaagacatatgaaaccactctagagaagtgctgtgccgctgcagatcctcatgaatgctatgccaaagtgttcgatgaatttaaacctcttgtggaagagcctcagaatttaatcaaacaaaattgtgagctttttgagcagcttggagagtacaaattccagaatgcgctattagttcgttacaccaagaaagtaccccaagtgtcaactccaactcttgtagaggtctcaagaaacctaggaaaagtgggcagcaaatgttgtaaacatcctgaagcaaaaagaatgccctgtgcagaagactatctatccgtggtcctgaaccagttatgtgtgttgcatgagaaaacgccagtaagtgacagagtcaccaaatgctgcacagaatccttggtgaacaggcgaccatgcttttcagctctggaagtcgatgaaacatacgttcccaaagagtttaatgctgaaacattcaccttccatgcagatatatgcacactttctgagaaggagagacaaatcaagaaacaaactgcacttgttgagcttgtgaaacacaagcccaaggcaacaaaagagcaactgaaagctgttatggatgatttcgcagcttttgtagagaagtgctgcaaggctgacgataaggagacctgctttgccgaggagggtaaaaaacttgttgctgcaagtcaagctgccttaggcttagcacctacttcaagttctacaaagaaaacacagctacaactggagcatttactgctggatttacagatgattttgaatggaattaataattacaagaatcccaaactcaccaggatgctcacatttaagttttacatgcccaagaaggccacagaactgaaacatcttcagtgtctagaagaagaactcaaacctctggaggaagtgctaaatttagctcaaagcaaaaactttcacttaagacccagggacttaatcagcaatatcaacgtaatagttctggaactaaagggatctgaaacaacattcatgtgtgaatatgctgatgagacagcaaccattgtagaatttctgaacagatggattaccttttgtcaaagcatcatctcaacactgacttgataa

SEQ ID NO: 3 - protein, 718 aa, rhIL-2/SA fusion, 9333
APTSSSTKKTQLQLEHLLLDLQMILNGINNYKNPKLTRMLTFKFYMPKKATELKHLQCLEEELKPLEEVLNLAQSKNFHLRPRDLISNINVIVLELKGSETTFMCEYADETATIVEFLNRWITFCQSIISTLTDAHKSEVAHRFKDLGEENFKALVLIAFAQYLQQCPFEDHVKLVNEVTEFAKTCVADESAENCDKSLHTLFGDKLCTVATLRETYGEMADCCAKQEPERNECFLQHKDDNPNLPRLVRPEVDVMCTAFHDNEETFLKKYLYEIARRHPYFYAPELLFFAKRYKAAFTECCQAADKAACLLPKLDELRDEGKASSAKQRLKCASLQKFGERAFKAWAVARLSQRFPKAEFAEVSKLVTDLTKVHTECCHGDLLECADDRADLAKYICENQDSISSKLKECCEKPLLEKSHCIAEVENDEMPADLPSLAADFVESKDVCKNYAEAKDVFLGMFLYEYARRHPDYSVVLLLRLAKTYETTLEKCCAAADPHECYAKVFDEFKPLVEEPQNLIKQNCELFEQLGEYKFQNALLVRYTKKVPQVSTPTLVEVSRNLGKVGSKCCKHPEAKRMPCAEDYLSVVLNQLCVLHEKTPVSDRVTKCCTESLVNRRPCFSALEVDETYVPKEFNAETFTFHADICTLSEKERQIKKQTALVELVKHKPKATKEQLKAVMDDFAAFVEKCCKADDKETCFAEEGKKLVAASQAALGL

SEQ ID NO: 4 - DNA, 2160 bp, rhIL-2/SA fusion, 9333
gctccaacttcctcatccactaagaaaacccagttgcagttggagcacttgttgttggacttgcagatgatcctgaacggtatcaacaactacaagaaccccaagctgaccagaatgctgaccttcaagttctacatgccaaagaaggccaccgagctgaagcacttgcaatgtttggaagaggaactgaagccactggaagaggttttgaacttggctcagtccaagaacttccacttgaggccaagagacttgatctccaacatcaacgtcatcgtcttggagttgaagggttccgagactaccttcatgtgtgaatacgctgacgagactgctaccatcgtcgagtttttgaacagatggatcaccttctgccagtccatcatctccactttgactgatgcacacaagagtgaggttgctcatcggtttaaagatttgggagaagaaaatttcaaagccttggtgttgattgcctttgctcagtatcttcagcagtgtccatttgaagatcatgtaaaattagtgaatgaagtaactgaatttgcaaaaacatgtgttgctgatgagtcagctgaaaattgtgacaaatcacttcataccctttttggagacaaattatgcacagttgcaactcttcgtgaaacctatggtgaaatggctgactgctgtgcaaaacaagaacctgagagaaatgaatgcttcttgcaacacaaagatgacaacccaaacctcccccgattggtgagaccagaggttgatgtgatgtgcactgcttttcatgacaatgaagagacatttttgaaaaaatacttatatgaaattgccagaagacatccttacttttatgccccggaactccttttctttgctaaaaggtataaagctgcttttacagaatgttgccaagctgctgataaagctgcctgcctgttgccaaagctcgatgaacttcgggatgaagggaaggcttcgtctgccaaacagagactcaagtgtgccagtctccaaaaatttggagaaagagctttcaaagcatgggcagtagctcgcctgagccagagatttcccaaagctgagtttgcagaagtttccaagttagtgacagatcttaccaaagtccacacggaatgctgccatggagatctgcttgaatgtgctgatgacagggcggaccttgccaagtatatctgtgaaaatcaagattcgatctccagtaaactgaaggaatgctgtgaaaaacctctgttggaaaaatcccactgcattgccgaagtggaaaatgatgagatgcctgctgacttgccttcattagctgctgattttgttgaaagtaaggatgtttgcaaaaactatgctgaggcaaaggatgtcttcctgggcatgtttttgtatgaatatgcaagaaggcatcctgattactctgtcgtgctgctgctgagacttgccaagacatatgaaaccactctagagaagtgctgtgccgctgcagatcctcatgaatgctatgccaaagtgttcgatgaatttaaacctcttgtggaagagcctcagaatttaatcaaacaaaattgtgagctttttgagcagcttggagagtacaaattccagaatgcgctattagttcgttacaccaagaaagtaccccaagtgtcaactccaactcttgtagaggtctcaagaaacctaggaaaagtgggcagcaaatgttgtaaacatcctgaagcaaaaagaatgccctgtgcagaagactatctatccgtggtcctgaaccagttatgtgtgttgcatgagaaaacgccagtaagtgacagagtcaccaaatgctgcacagaatccttggtgaacaggcgaccatgcttttcagctctggaagtcgatgaaacatacgttcccaaagagtttaatgctgaaacattcaccttccatgcagatatatgcacactttctgagaaggagagacaaatcaagaaacaaactgcacttgttgagcttgtgaaacacaagcccaaggcaacaaaagagcaactgaaagctgttatggatgatttcgcagcttttgtagagaagtgctgcaaggctgacgataaggagacctgctttgccgaggagggtaaaaaacttgttgctgcaagtcaagctgccttaggcttatgataa

SEQ ID NO: 5 - protein, 718 aa, rhIL-2v5/SA fusion, 9555
APASSSTKKTQLQLEHLLLDLQMILNGINNYKNPKLTRMLTAKFAMPKKATELKHLQCLEEELKPLEEVLNGAQSKNFHLRPRDLISNINVIVLELKGSETTFMCEYADETATIVEFLNRWITFAQSIISTLTDAHKSEVAHRFKDLGEENFKALVLIAFAQYLQQCPFEDHVKLVNEVTEFAKTCVADESAENCDKSLHTLFGDKLCTVATLRETYGEMADCCAKQEPERNECFLQHKDDNPNLPRLVRPEVDVMCTAFHDNEETFLKKYLYEIARRHPYFYAPELLFFAKRYKAAFTECCQAADKAACLLPKLDELRDEGKASSAKQRLKCASLQKFGERAFKAWAVARLSQRFPKAEFAEVSKLVTDLTKVHTECCHGDLLECADDRADLAKYICENQDSISSKLKECCEKPLLEKSHCIAEVENDEMPADLPSLAADFVESKDVCKNYAEAKDVFLGMFLYEYARRHPDYSVVLLLRLAKTYETTLEKCCAAADPHECYAKVFDEFKPLVEEPQNLIKQNCELFEQLGEYKFQNALLVRYTKKVPQVSTPTLVEVSRNLGKVGSKCCKHPEAKRMPCAEDYLSVVLNQLCVLHEKTPVSDRVTKCCTESLVNRRPCFSALEVDETYVPKEFNAETFTFHADICTLSEKERQIKKQTALVELVKHKPKATKEQLKAVMDDFAAFVEKCCKADDKETCFAEEGKKLVAASQAALGL

SEQ ID NO: 6 - DNA, 2160 bp, rhIL-2v5/SA fusion, 9555
gctccagcttcctcatccactaagaaaacccagttgcagttggagcacttgttgttggacttgcagatgatcctgaacggtatcaacaactacaagaaccccaagctgaccagaatgctgaccgctaagttcgctatgccaaagaaggccaccgagctgaagcacttgcaatgtttggaagaggaactgaagccactggaagaggttttgaacggtgctcagtccaagaacttccacttgaggccaagagacttgatctccaacatcaacgtcatcgtcttggagttgaagggttccgagactaccttcatgtgtgaatacgctgacgagactgctaccatcgtcgagtttttgaacagatggatcaccttcgctcagtccatcatctccactttgactgatgcacacaagagtgaggttgctcatcggtttaaagatttgggagaagaaaatttcaaagccttggtgttgattgcctttgctcagtatcttcagcagtgtccatttgaagatcatgtaaaattagtgaatgaagtaactgaatttgcaaaaacatgtgttgctgatgagtcagctgaaaattgtgacaaatcacttcataccctttttggagacaaattatgcacagttgcaactcttcgtgaaacctatggtgaaatggctgactgctgtgcaaaacaagaacctgagagaaatgaatgcttcttgcaacacaaagatgacaacccaaacctcccccgattggtgagaccagaggttgatgtgatgtgcactgcttttcatgacaatgaagagacatttttgaaaaaatacttatatgaaattgccagaagacatccttacttttatgccccggaactccttttctttgctaaaaggtataaagctgcttttacagaatgttgccaagctgctgataaagctgcctgcctgttgccaaagctcgatgaacttcgggatgaagggaaggcttcgtctgccaaacagagactcaagtgtgccagtctccaaaaatttggagaaagagctttcaaagcatgggcagtagctcgcctgagccagagatttcccaaagctgagtttgcagaagtttccaagttagtgacagatcttaccaaagtccacacggaatgctgccatggagatctgcttgaatgtgctgatgacagggcggaccttgccaagtatatctgtgaaaatcaagattcgatctccagtaaactgaaggaatgctgtgaaaaacctctgttggaaaaatcccactgcattgccgaagtggaaaatgatgagatgcctgctgacttgccttcattagctgctgattttgttgaaagtaaggatgtttgcaaaaactatgctgaggcaaaggatgtcttcctgggcatgtttttgtatgaatatgcaagaaggcatcctgattactctgtcgtgctgctgctgagacttgccaagacatatgaaaccactctagagaagtgctgtgccgctgcagatcctcatgaatgctatgccaaagtgttcgatgaatttaaacctcttgtggaagagcctcagaatttaatcaaacaaaattgtgagctttttgagcagcttggagagtacaaattccagaatgcgctattagttcgttacaccaagaaagtaccccaagtgtcaactccaactcttgtagaggtctcaagaaacctaggaaaagtgggcagcaaatgttgtaaacatcctgaagcaaaaagaatgccctgtgcagaagactatctatccgtggtcctgaaccagttatgtgtgttgcatgagaaaacgccagtaagtgacagagtcaccaaatgctgcacagaatccttggtgaacaggcgaccatgcttttcagctctggaagtcgatgaaacatacgttcccaaagagtttaatgctgaaacattcaccttccatgcagatatatgcacactttctgagaaggagagacaaatcaagaaacaaactgcacttgttgagcttgtgaaacacaagcccaaggcaacaaaagagcaactgaaagctgttatggatgatttcgcagcttttgtagagaagtgctgcaaggctgacgataaggagacctgctttgccgaggagggtaaaaaacttgttgctgcaagtcaagctgccttaggcttatgataa

SEQ ID NO: 7 - protein, 718 aa, rHSA/IL-2v7 fusion, 9777
DAHKSEVAHRFKDLGEENFKALVLIAFAQYLQQCPFEDHVKLVNEVTEFAKTCVADESAENCDKSLHTLFGDKLCTVATLRETYGEMADCCAKQEPERNECFLQHKDDNPNLPRLVRPEVDVMCTAFHDNEETFLKKYLYEIARRHPYFYAPELLFFAKRYKAAFTECCQAADKAACLLPKLDELRDEGKASSAKQRLKCASLQKFGERAFKAWAVARLSQRFPKAEFAEVSKLVTDLTKVHTECCHGDLLECADDRADLAKYICENQDSISSKLKECCEKPLLEKSHCIAEVENDEMPADLPSLAADFVESKDVCKNYAEAKDVFLGMFLYEYARRHPDYSVVLLLRLAKTYETTLEKCCAAADPHECYAKVFDEFKPLVEEPQNLIKQNCELFEQLGEYKFQNALLVRYTKKVPQVSTPTLVEVSRNLGKVGSKCCKHPEAKRMPCAEDYLSVVLNQLCVLHEKTPVSDRVTKCCTESLVNRRPCFSALEVDETYVPKEFNAETFTFHADICTLSEKERQIKKQTALVELVKHKPKATKEQLKAVMDDFAAFVEKCCKADDKETCFAEEGKKLVAASQAALGLAPASSSTKKTQLQLEHLLLDLQMILNGINNYKNPKLTAMLTAKFAMPKKATELKHLQCLEEALKPLEEVLNGAQSKNFHLRPRDLISNINVIVLELKGSETTFMCEYADETATIVEFLNRWITFAQSIISTLT

SEQ ID NO: 8 - DNA, 2232 bp, rHSA/IL-2v7 fusion, 9777
atgaagtgggtaacctttatttcccttctttttctctttagctcggcttattccaggggtgtgtttcgtcgagatgcacacaagagtgaggttgctcatcggtttaaagatttgggagaagaaaatttcaaagccttggtgttgattgcctttgctcagtatcttcagcagtgtccatttgaagatcatgtaaaattagtgaatgaagtaactgaatttgcaaaaacatgtgttgctgatgagtcagctgaaaattgtgacaaatcacttcataccctttttggagacaaattatgcacagttgcaactcttcgtgaaacctatggtgaaatggctgactgctgtgcaaaacaagaacctgagagaaatgaatgcttcttgcaacacaaagatgacaacccaaacctcccccgattggtgagaccagaggttgatgtgatgtgcactgcttttcatgacaatgaagagacatttttgaaaaaatacttatatgaaattgccagaagacatccttacttttatgccccggaactccttttctttgctaaaaggtataaagctgcttttacagaatgttgccaagctgctgataaagctgcctgcctgttgccaaagctcgatgaacttcgggatgaagggaaggcttcgtctgccaaacagagactcaagtgtgccagtctccaaaaatttggagaaagagctttcaaagcatgggcagtagctcgcctgagccagagatttcccaaagctgagtttgcagaagtttccaagttagtgacagatcttaccaaagtccacacggaatgctgccatggagatctgcttgaatgtgctgatgacagggcggaccttgccaagtatatctgtgaaaatcaagattcgatctccagtaaactgaaggaatgctgtgaaaaacctctgttggaaaaatcccactgcattgccgaagtggaaaatgatgagatgcctgctgacttgccttcattagctgctgattttgttgaaagtaaggatgtttgcaaaaactatgctgaggcaaaggatgtcttcctgggcatgtttttgtatgaatatgcaagaaggcatcctgattactctgtcgtgctgctgctgagacttgccaagacatatgaaaccactctagagaagtgctgtgccgctgcagatcctcatgaatgctatgccaaagtgttcgatgaatttaaacctcttgtggaagagcctcagaatttaatcaaacaaaattgtgagctttttgagcagcttggagagtacaaattccagaatgcgctattagttcgttacaccaagaaagtaccccaagtgtcaactccaactcttgtagaggtctcaagaaacctaggaaaagtgggcagcaaatgttgtaaacatcctgaagcaaaaagaatgccctgtgcagaagactatctatccgtggtcctgaaccagttatgtgtgttgcatgagaaaacgccagtaagtgacagagtcaccaaatgctgcacagaatccttggtgaacaggcgaccatgcttttcagctctggaagtcgatgaaacatacgttcccaaagagtttaatgctgaaacattcaccttccatgcagatatatgcacactttctgagaaggagagacaaatcaagaaacaaactgcacttgttgagcttgtgaaacacaagcccaaggcaacaaaagagcaactgaaagctgttatggatgatttcgcagcttttgtagagaagtgctgcaaggctgacgataaggagacctgctttgccgaggagggtaaaaaacttgttgctgcaagtcaagctgccttaggcttagctccagcttcctcatccactaagaaaacccagttgcagttggagcacttgttgttggacttgcagatgatcctgaacggtatcaacaactacaagaaccccaagctgaccgctatgctgaccgctaagttcgctatgccaaagaaggccaccgagctgaagcacttgcaatgtttggaagaggctctgaagccactggaagaggttttgaacggtgctcagtccaagaacttccacttgaggccaagagacttgatctccaacatcaacgtcatcgtcttggagttgaagggttccgagactaccttcatgtgtgaatacgctgacgagactgctaccatcgtcgagtttttgaacagatggatcaccttcgctcagtccatcatctccactttgacttgataa

SEQ ID NO: 9 - protein, 585 aa, Human Serum Albumin mature protein [sequence omitted]

SEQ ID NO: 10 - protein, 133 aa, Human Interleukin-2 mature protein, wild-type [sequence omitted]

SEQ ID NO: 11 - DNA, 30 bp, Human Serum Albumin PCR primer-1
gaattcatgaagtgggtaacctttatttcc

SEQ ID NO: 12 - DNA, 33 bp, Human Serum Albumin PCR primer-2
gaattcttataagcctaaggcagcttgacttgc

SEQ ID NO: 13 - DNA, 19 bp, albumin-IL-2 fusion protein sequence primer-P1
ctggttccaattgacaagc

SEQ ID NO: 14 - DNA, 19 bp, albumin-IL-2 fusion protein sequence primer-P9
gactcatcagcaacacatg